European Patent Specification EP 3 516 064 B1, published April 16, 2025. Title: New Promoters. Applicant: Boehringer Ingelheim Vetmedica GmbH. The sequence listing filed with the application follows.

SEQUENCE LISTING (37 sequences)

SEQ ID NO: 1 - DNA, 600 bp, Equine herpesvirus 4
gcagactttggagcagcacaatttccggttgtggaccccatggaccttggtttggctggtaccgtggaaactaacgctccggaagttttggccagagcaaaatacaattcgaaggtagacatatggagcgccggaatagttctgtttgaaatgctcgcatatccatcaactctatttgaggacccgccgagtaccccacaagagtatgtaaaaagctgtcattctcaactactgagaataatatcaaagctaaagataaaccctgaggagtttccacgggaaccagagtctaggctcgtgcgcggatacatcgaatacgccagcctagagcgtaagccacatacgcgctatccttgcttccagcgcgtgaacctacacattgacggggaatttttgatccataaaatgctagcgttcaatgctgcgatgcgcccatccgcagaagagttgttgtcctacccaatgtttatgaatctgtaggatgactaacagatttggggtggagacggcgtgggcgatactgtataaagttgtactacttaccagcccagtcagtgtgctgtagtgccaccacctgtaaagctgtgataagctgcagtt

SEQ ID NO: 2 - DNA, 600 bp, Equine herpesvirus 4
agctgggggagtttgtactatagtgtattacatgcggcttgcaataactgcctggtttatgtttcgcaacattcaagcagacatgctaccgctaaacactttgcaacaattttttattgggtgtttggcctttggtagaactgtcgcgtttttggtggtagcatatactaccttatttatacgctccgagctgtttttcagcatgctagcacccaacgccgagcgagagtatataactcccatcattgcccacaagcttatgccacttattagcgtccgctctgccgtttgcttagtcataatatctaccgccgtttacgcagcagacgctatctgcgacacaattggatttgcgataccgcgcatgtggatgtgtattttaatgagatcaacctccatgaagcgtaactagggggcctcccactgaggcactaccggcttagcagctgactaacacagtataaaacgtgagaagaaatcagtctcatgcgccattagcgctaggctagttagcgtggaggaccggagcgctaccgccagcagtttcatccgcctggttacgggtttgttaacacctaccggtgttttaccgctaccata

SEQ ID NO: 3 - DNA, 430 bp, Equine herpesvirus 4
tctatttgaggacccgccgagtaccccacaagagtatgtaaaaagctgtcattctcaactactgagaataatatcaaagctaaagataaaccctgaggagtttccacgggaaccagagtctaggctcgtgcgcggatacatcgaatacgccagcctagagcgtaagccacatacgcgctatccttgcttccagcgcgtgaacctacacattgacggggaatttttgatccataaaatgctagcgttcaatgctgcgatgcgcccatccgcagaagagttgttgtcctacccaatgtttatgaatctgtaggatgactaacagatttggggtggagacggcgtgggcgatactgtataaagttgtactacttaccagcccagtcagtgtgctgtagtgccaccacctgtaaagctgtgataagctgcagtt

SEQ ID NO: 4 - DNA, 449 bp, Equine herpesvirus 4
ttggtggtagcatatactaccttatttatacgctccgagctgtttttcagcatgctagcacccaacgccgagcgagagtatataactcccatcattgcccacaagcttatgccacttattagcgtccgctctgccgtttgcttagtcataatatctaccgccgtttacgcagcagacgctatctgcgacacaattggatttgcgataccgcgcatgtggatgtgtattttaatgagatcaacctccatgaagcgtaactagggggcctcccactgaggcactaccggcttagcagctgactaacacagtataaaacgtgagaagaaatcagtctcatgcgccattagcgctaggctagttagcgtggaggaccggagcgctaccgccagcagtttcatccgcctggttacgggtttgttaacacctaccggtgttttaccgctaccata

SEQ ID NO: 5 - DNA, 20 bp, Artificial Sequence
  primer no 1130 specific for orf72
tgtctaccttcaagcttatg

SEQ ID NO: 6 - DNA, 17 bp, Artificial Sequence
  primer no 1131 specific for orf72
ctagcgcagtcgcgttg

SEQ ID NO: 7 - DNA, 18 bp, Artificial Sequence
  primer no. 1079 specific for mCherry
gcgaggaggataacatgg

SEQ ID NO: 8 - DNA, 18 bp, Artificial Sequence
  primer no. 1080 specific for mCherry
acccttggtcaccttcag

SEQ ID NO: 9 - DNA, 22 bp, Artificial Sequence
  Artificial sequence nucleic acid PCR primer 1017 for the orf70 insertion region
aggctcgtgcgcggatacatcg

SEQ ID NO: 10 - DNA, 22 bp, Artificial Sequence
  Artificial sequence nucleic acid PCR primer 1018 for the orf70 insertion region
ttcggggctgttagactcctcc

SEQ ID NO: 11 - DNA, 22 bp, Artificial Sequence
  Artificial sequence nucleic acid PCR primer 1007 for the orf1/3 insertion region
ccaactcgccgccatgagaccc

SEQ ID NO: 12 - DNA, 22 bp, Artificial Sequence
  Artificial sequence nucleic acid PCR primer 1008 for the orf1/3 insertion region
agcgcgccccgtacccagtggg

SEQ ID NO: 13 - DNA, 417 bp, Equine herpesvirus 1
ctccgagtaccccagaggagtatgtgaaaagctgccactcgcaactactgaagataatttcaacgctcaagataaatccggaggagtttcctcgagaccccgggtcgaggctcgtgcgcggatacatcgagtattctagactcgagcgcaagccctacacgcgctacccctgctttcaacgcgtcaacctgcacattgacggggagtttctggttcacaagatgctagcgttcaatgccgcgatgcgcccatcggccgaggagctgctgtcatacccaatgtttgctcaactttaggatgactaacctgtttctgggaggagacagcgtgggcgacggtgtataaagttggtctgctttcaagccctgccactgcgctacagtgccaccaactgtaaagcggtagtaagctgcagtg

SEQ ID NO: 14 - DNA, 431 bp, Equine herpesvirus 1
gaccctgttggtgggtgcggttggactcagaatcttggcgcaggcatggaagtttgtcggtgacgaaacatacgacaccatccgcgcagaagcaaagaatttagagacccacgtaccctcaagtgctgcagagtcgtctctagaaaaccaatcgacacaggaggagtctaacagccccgaagttgcccacctgcgaagcgtcaacagcgatgacagtacacacacggggggtgcgtcgaacggcatccaggactgtgacagtcagctcaaaactgtgtatgcctgcttggctctaattggactcggcacatgtgccatgatagggttgatagtttacatttgtgtattaaggtcaaaactgtcctctcggaatttttcgcgcgcgcaaaatgtaaaacatagaaattaccagcgacttgagtacgttgctt

SEQ ID NO: 15 - DNA, 417 bp, Equine herpesvirus 1
ctccgagtaccccagaggagtatgtgaaaagctgccactcgcaactactgaagataatttcaacgctcaagataaatccggaggagtttcctcgagaccccgggtcgaggctcgtgcgcggatacatcgagtattctagactcgagcgcaagccctacacgcgctacccctgctttcaacgcgtcaacctgcacattgacggggagtttctggttcacaagatgctagcgttcaatgccgcgatgcgcccatcggccgaggagctgctgtcatacccaatgtttgcacaactttaggatgactaacctgtttctgggaggagacagcgtgggcgacggtgtataaagttggtctgctttcaagccctgccactgcgctacagtgccaccaactgtaaagcggtagtaagctgcagtg

SEQ ID NO: 16 - DNA, 431 bp, Equine herpesvirus 1; identical to SEQ ID NO: 14

SEQ ID NO: 17 - DNA, 283 bp, Equine herpesvirus 1
tctagactcgagcgcaagccctacacgcgctacccctgctttcaacgcgtcaacctgcacattgacggggagtttctggttcacaagatgctagcgttcaatgccgcgatgcgcccatcggccgaggagctgctgtcatacccaatgtttgctcaactttaggatgactaacctgtttctgggaggagacagcgtgggcgacggtgtataaagttggtctgctttcaagccctgccactgcgctacagtgccaccaactgtaaagcggtagtaagctgcagtg

SEQ ID NO: 18 - DNA, 144 bp, Equine herpesvirus 1
gaccctgttggtgggtgcggttggactcagaatcttggcgcaggcatggaagtttgtcggtgacgaaacatacgacaccatccgcgcagaagcaaagaatttagagacccacgtaccctcaagtgctgcagagtcgtctctaga

SEQ ID NO: 19 - DNA, 801 bp, Equine herpesvirus 1
atgttgactgtcttagcagccctgagtctgctcagcttgcttacgagcgcaaccggacggctcgccccagatgaactctgttatgccgaaccccgcagaactggcagcccaccaaacacccagcccgaacgcccacccgtaatatttgagcccccaacaattgcgattaaagctgaatccaagggttgtgagctaattttattagatccacccatagatgtaagctatcgcagagaagataaggtgaatgcgtccattgcttggttttttgactttggcgcttgccggatgcccatcgcatacagagagtattacggttgtattggcaatgctgttccctccccagagacttgtgatgcgtactcatttacccttattaggaccgagggtatcgtggagtttaccatcgtaaacatgagcctcctgtttcagcctggaatatacgatagtggcaattttatctacagcgttctcctggactaccacatatttacaggacgtgtaacgttggaagtggaaaaggacacaaactatccctgtggcatgattcatggactcactgcttacggaaacatcaacgtagatgaaaccatggacaacgccagcccacacccgcgtgccgtggggtgctttcccgagcccatcgacaacgaagcgtgggcaaacgttacatttactgaattggggataccagacccaaactcatttctcgatgacgagggtgattacccgaatatatcagactgtcactcgtgggagtcatacacctacccaaatacgctgaggcaggccacaggaccc

SEQ ID NO: 20 - DNA, 801 bp, Equine herpesvirus 1
atgttgactgtcttagcagctctgagtctgctcagcttgcttacgagcgcaaccggacggctcgccccagatgaactctgttatgccgaaccccgcagaactggcagcccaccaaacacccagcccgaacgcccacccgtaatatttgagcccccaacaattgcgattaaagctgaatccaagggttgtgagctaattttattagatccacccatagatgtaagctatcgcagagaagataaggtgaatgcgtccattgcttggttttttgactttggcgcttgccggatgcccatcgcatacagagagtattacggttgtattggcaatgctgttccctccccagagacttgtgatgcgtactcatttacccttattaggaccgagggtatcgtggagtttaccatcgtaaacatgagcctcctgtttcagcctggaatatacgatagtggcaattttatctacagcgttctcctggactaccacatatttacaggacgtgtaacgttggaagtggaaaaggacacaaactatccctgtggcatgattcatggactcactgcttacggaaacatcaacgtagatgaaaccatggacaacgccagcccacacccgcgtgccgtggggtgctttcccgagcccatcgacaacgaagcgtgggcaaacgttacatttactgaattggggataccagacccaaactcatttctcgatgacgagggtgattacccgaatatatcagactgtcactcgtgggagtcatacacctacccaaatacgctgaggcaggccacaggaccc

SEQ ID NO: 21 - DNA, 4435 bp, Artificial Sequence
  Nucleotide sequence of transfer plasmid pU-mC70-BGH
tcgcgcgtttcggtgatgacggtgaaaacctctgacacatgcagctcccggagacggtcacagcttgtctgtaagcggatgccgggagcagacaagcccgtcagggcgcgtcagcgggtgttggcgggtgtcggggctggcttaactatgcggcatcagagcagattgtactgagagtgcaccatatgcggtgtgaaataccgcacagatgcgtaaggagaaaataccgcatcaggcgccattcgccattcaggctgcgcaactgttgggaagggcgatcggtgcgggcctcttcgctattacgccagctggcgaaagggggatgtgctgcaaggcgattaagttgggtaacgccagggttttcccagtcacgacgttgtaaaacgacggccagtgaattcctccgagtaccccagaggagtatgtgaaaagctgccactcgcaactactgaagataatttcaacgctcaagataaatccggaggagtttcctcgagaccccgggtcgaggctcgtgcgcggatacatcgagtattctagactcgagcgcaagccctacacgcgctacccctgctttcaacgcgtcaacctgcacattgacggggagtttctggttcacaagatgctagcgttcaatgccgcgatgcgcccatcggccgaggagctgctgtcatacccaatgtttgctcaactttaggatgactaacctgtttctgggaggagacagcgtgggcgacggtgtataaagttggtctgctttcaagccctgccactgcgctacagtgccaccaactgtaaagcggtagtaagctgcagtggtcgacatggtgagcaagggcgaggaggataacatggccatcatcaaggagttcatgcgcttcaaggtgcacatggagggctccgtgaacggccacgagttcgagatcgagggcgagggcgagggccgcccctacgagggcacccagaccgccaagctgaaggtgaccaagggtggccccctgcccttcgcctgggacatcctgtcccctcagttcatgtacggctccaaggcctacgtgaagcaccccgccgacatccccgactacttgaagctgtccttccccgagggcttcaagtgggagcgcgtgatgaacttcgaggacggcggcgtggtgaccgtgacccaggactcctccctgcaggacggcgagttcatctacaaggtgaagctgcgcggcaccaacttcccctccgacggccccgtaatgcagaagaagaccatgggctgggaggcctcctccgagcggatgtaccccgaggacggcgccctgaagggcgagatcaagcagaggctgaagctgaaggacggcggccactacgacgctgaggtcaagaccacctacaaggccaagaagcccgtgcagctgcccggcgcctacaacgtcaacatcaagttggacatcacctcccacaacgaggactacaccatcgtggaacagtacgaacgcgccgagggccgccactccaccggcggcatggacgagctgtacaagtaactgtgccttctagttgccagccatctgttgtttgcccctcccccgtgccttccttgaccctggaaggtgccactcccactgtcctttcctaataaaatgaggaaattgcatcgcattgtctgagtaggtgtcattctattctggggggtggggtggggcaggacagcaagggggaggattgggaagacaatagcaggcatgctggggatgcggtgggctctatggatccgaccctgttggtgggtgcggttggactcagaatcttggcgcaggcatggaagtttgtcggtgacgaaacatacgacaccatccgcgcagaagcaaagaatttagagacccacgtaccctcaagtgctgcagagtcgtctctagaaaaccaatcgacacaggaggagtctaacagccccgaagttgcccacctgcgaagcgtcaacagcgatgacagtacacacacggggggtgcgtcgaacggcatccaggactgtgacagtcagctcaaaactgtgtatgcctgcttggctctaattggactcggcacatgtgccatgatagggttgatagtttacatttgtgtattaaggtcaaaactgtcctctcggaatttttcgcgcgcgcaaaatgtaaaacatagaaattaccagcgacttgagtacgttgcttaagcttggcgtaatcatggtcatagctgtttcctgtgtgaaattgttatccgctcacaattccacacaacatacgagccggaagcataaagtgtaaagcctggggtgcctaatgagtgagctaactcacattaattgcgttgcgctcactgcccgctttccagtcgggaaacctgtcgtgccagctgcattaatgaatcggccaacgcgcggggagaggcggtttgcgtattgggcgctcttccgcttcctcgctcactgactcgctgcgctcggtcgttcggctgcggcgagcggtatcagctcactcaaaggcggtaatacggttatccacagaatcaggggataacgcaggaaagaacatgtgagcaaaaggccagcaaaaggccaggaaccgtaaaaaggccgcgttgctggcgtttttccataggctccgcccccctgacgagcatcacaaaaatcgacgctcaagtcagaggtggcgaaacccgacaggactataaagataccaggcgtttccccctggaagctccctcgtgcgctctcctgttccgaccctgccgcttaccggatacctgtccgcctttctcccttcgggaagcgtggcgctttctcatagctcacgctgtaggtatctcagttcggtgtaggtcgttcgctccaagctgggctgtgtgcacgaaccccccgttcagcccgaccgctgcgccttatccggtaactatcgtcttgagtccaacccggtaagacacgacttatcgccactggcagcagccactggtaacaggattagcagagcgaggtatgtaggcggtgctacagagttcttgaagtggtggcctaactacggctacactagaaggacagtatttggtatctgcgctctgctgaagccagttaccttcggaaaaagagttggtagctcttgatccggcaaacaaaccaccgctggtagcggtggtttttttgtttgcaagcagcagattacgcgcagaaaaaaaggatctcaagaagatcctttgatcttttctacggggtctgacgctcagtggaacgaaaactcacgttaagggattttggtcatgagattatcaaaaaggatcttcacctagatccttttaaattaaaaatgaagttttaaatcaatctaaagtatatatgagtaaacttggtctgacagttaccaatgcttaatcagtgaggcacctatctcagcgatctgtctatttcgttcatccatagttgcctgactccccgtcgtgtagataactacgatacgggagggcttaccatctggccccagtgctgcaatgataccgcgagacccacgctcaccggctccagatttatcagcaataaaccagccagccggaagggccgagcgcagaagtggtcctgcaactttatccgcctccatccagtctattaattgttgccgggaagctagagtaagtagttcgccagttaatagtttgcgcaacgttgttgccattgctacaggcatcgtggtgtcacgctcgtcgtttggtatggcttcattcagctccggttcccaacgatcaaggcgagttacatgatcccccatgttgtgcaaaaaagcggttagctccttcggtcctccgatcgttgtcagaagtaagttggccgcagtgttatcactcatggttatggcagcactgcataattctcttactgtcatgccatccgtaagatgcttttctgtgactggtgagtactcaaccaagtcattctgagaatagtgtatgcggcgaccgagttgctcttgcccggcgtcaatacgggataataccgcgccacatagcagaactttaaaagtgctcatcattggaaaacgttcttcggggcgaaaactctcaaggatcttaccgctgttgagatccagttcgatgtaacccactcgtgcacccaactgatcttcagcatcttttactttcaccagcgtttctgggtgagcaaaaacaggaaggcaaaatgccgcaaaaaagggaataagggcgacacggaaatgttgaatactcatactcttcctttttcaatattattgaagcatttatcagggttattgtctcatgagcggatacatatttgaatgtatttagaaaaataaacaaataggggttccgcgcacatttccccgaaaagtgccacctgacgtctaagaaaccattattatcatgacattaacctataaaaataggcgtatcacgaggccctttcgtc

SEQ ID NO: 22 - DNA, 5191 bp, Artificial Sequence
  Nucleotide sequence of transfer vector pU70-p455-71K71
caataaacgcggtatgtctaccttcaagcctatgatgaacggatgtttggtgtttgcggctattataacgctcttgagttttatgctatctctgggaacatgcgaaaattacaggcgtgtggttcgggatcctagggataacagggtaatcgatttattcaacaaagccacgttgtgtctcaaaatctctgatgttacattgcacaagataaaaatatatcatcatgaacaataaaactgtctgcttacataaacagtaatacaaggggtgttatgagccatattcaacgggaaacgtcttgctcgaggccgcgattaaattccaacatggatgctgatttatatgggtataaatgggctcgcgataatgtcgggcaatcaggtgcgacaatctatcgattgtatgggaagcccgatgcgccagagttgtttctgaaacatggcaaaggtagcgttgccaatgatgttacagatgagatggtcagactaaactggctgacggaatttatgcctcttccgaccatcaagcattttatccgtactcctgatgatgcatggttactcaccactgcgatccccgggaaaacagcattccaggtattagaagaatatcctgattcaggtgaaaatattgttgatgcgctggcagtgttcctgcgccggttgcattcgattcctgtttgtaattgtccttttaacagcgatcgcgtatttcgtctcgctcaggcgcaatcacgaatgaataacggtttggttgatgcgagtgattttgatgacgagcgtaatggctggcctgttgaacaagtctggaaagaaatgcataagcttttgccattctcaccggattcagtcgtcactcatggtgatttctcacttgataaccttatttttgacgaggggaaattaataggttgtattgatgttggacgagtcggaatcgcagaccgataccaggatcttgccatcctatggaactgcctcggtgagttttctccttcattacagaaacggctttttcaaaaatatggtattgataatcctgatatgaataaattgcagtttcatttgatgctcgatgagtttttctaaaataaacgcggtatgtctaccttcaagcctatgatgaacggatgtttggtgtttgcggctattataacgctcttgagttttatgctatctctgggaacatgcgaaaattacaggcgtgtggttcgggatccgaccctgttggtgggtgcggttggactcagaatcttggcgcaggcatggaagtttgtcggtgacgaaacatacgacaccatccgcgcagaagcaaagaatttagagacccacgtaccctcaagtgctgcagagtcgtctctagaaaaccaatcgacacaggaggagtctaacagccccgaagttgcccacctgcgaagcgtcaacagcgatgacagtacacacacggggggtgcgtcgaacggcatccaggactgtgacagtcagctcaaaactgtgtatgcctgcttggctctaattggactcggcacatgtgccatgatagggttgatagtttacatttgtgtattaaggtcaaaactgtcctctcggaatttttcgcgcgcgcaaaatgtaaaacatagaaattaccagcgacttgagtacgttgcttaagcttggcgtaatcatggtcatagctgtttcctgtgtgaaattgttatccgctcacaattccacacaacatacgagccggaagcataaagtgtaaagcctggggtgcctaatgagtgagctaactcacattaattgcgttgcgctcactgcccgctttccagtcgggaaacctgtcgtgccagctgcattaatgaatcggccaacgcgcggggagaggcggtttgcgtattgggcgctcttccgcttcctcgctcactgactcgctgcgctcggtcgttcggctgcggcgagcggtatcagctcactcaaaggcggtaatacggttatccacagaatcaggggataacgcaggaaagaacatgtgagcaaaaggccagcaaaaggccaggaaccgtaaaaaggccgcgttgctggcgtttttccataggctccgcccccctgacgagcatcacaaaaatcgacgctcaagtcagaggtggcgaaacccgacaggactataaagataccaggcgtttccccctggaagctccctcgtgcgctctcctgttccgaccctgccgcttaccggatacctgtccgcctttctcccttcgggaagcgtggcgctttctcatagctcacgctgtaggtatctcagttcggtgtaggtcgttcgctccaagctgggctgtgtgcacgaaccccccgttcagcccgaccgctgcgccttatccggtaactatcgtcttgagtccaacccggtaagacacgacttatcgccactggcagcagccactggtaacaggattagcagagcgaggtatgtaggcggtgctacagagttcttgaagtggtggcctaactacggctacactagaaggacagtatttggtatctgcgctctgctgaagccagttaccttcggaaaaagagttggtagctcttgatccggcaaacaaaccaccgctggtagcggtggtttttttgtttgcaagcagcagattacgcgcagaaaaaaaggatctcaagaagatcctttgatcttttctacggggtctgacgctcagtggaacgaaaactcacgttaagggattttggtcatgagattatcaaaaaggatcttcacctagatccttttaaattaaaaatgaagttttaaatcaatctaaagtatatatgagtaaacttggtctgacagttaccaatgcttaatcagtgaggcacctatctcagcgatctgtctatttcgttcatccatagttgcctgactccccgtcgtgtagataactacgatacgggagggcttaccatctggccccagtgctgcaatgataccgcgagacccacgctcaccggctccagatttatcagcaataaaccagccagccggaagggccgagcgcagaagtggtcctgcaactttatccgcctccatccagtctattaattgttgccgggaagctagagtaagtagttcgccagttaatagtttgcgcaacgttgttgccattgctacaggcatcgtggtgtcacgctcgtcgtttggtatggcttcattcagctccggttcccaacgatcaaggcgagttacatgatcccccatgttgtgcaaaaaagcggttagctccttcggtcctccgatcgttgtcagaagtaagttggccgcagtgttatcactcatggttatggcagcactgcataattctcttactgtcatgccatccgtaagatgcttttctgtgactggtgagtactcaaccaagtcattctgagaatagtgtatgcggcgaccgagttgctcttgcccggcgtcaatacgggataataccgcgccacatagcagaactttaaaagtgctcatcattggaaaacgttcttcggggcgaaaactctcaaggatcttaccgctgttgagatccagttcgatgtaacccactcgtgcacccaactgatcttcagcatcttttactttcaccagcgtttctgggtgagcaaaaacaggaaggcaaaatgccgcaaaaaagggaataagggcgacacggaaatgttgaatactcatactcttcctttttcaatattattgaagcatttatcagggttattgtctcatgagcggatacatatttgaatgtatttagaaaaataaacaaataggggttccgcgcacatttccccgaaaagtgccacctgacgtctaagaaaccattattatcatgacattaacctataaaaataggcgtatcacgaggccctttcgtctcgcgcgtttcggtgatgacggtgaaaacctctgacacatgcagctcccggagacggtcacagcttgtctgtaagcggatgccgggagcagacaagcccgtcagggcgcgtcagcgggtgttggcgggtgtcggggctggcttaactatgcggcatcagagcagattgtactgagagtgcaccatatgcggtgtgaaataccgcacagatgcgtaaggagaaaataccgcatcaggcgccattcgccattcaggctgcgcaactgttgggaagggcgatcggtgcgggcctcttcgctattacgccagctggcgaaagggggatgtgctgcaaggcgattaagttgggtaacgccagggttttcccagtcacgacgttgtaaaacgacggccagtgaattcctccgagtaccccagaggagtatgtgaaaagctgccactcgcaactactgaagataatttcaacgctcaagataaatccggaggagtttcctcgagaccccgggtcgaggctcgtgcgcggatacatcgagtattctagactcgagcgcaagccctacacgcgctacccctgctttcaacgcgtcaacctgcacattgacggggagtttctggttcacaagatgctagcgttcaatgccgcgatgcgcccatcggccgaggagctgctgtcatacccaatgtttgctcaactttaggatgactaacctgtttctgggaggagacagcgtgggcgacggtgtataaagttggtctgctttcaagccctgccactgcgctacagtgccaccaactgtaaagcggtagtaagctgcagtggtcgactggtggtagcatatactaccttatttatacgctccgagctgtttttcagcatgctagcacccaacgccgagcgagagtatataactcccatcattgcccacaagcttatgccacttattagcgtccgctctgccgtttgcttagtcataatatctaccgccgtttacgcagcagacgctatctgcgacacaattggatttgcgataccgcgcatgtggatgtgtattttaatgagatcaacctccatgaagcgtaactagggggcctcccactgaggcactaccggcttagcagctgactaacacagtataaaacgtgagaagaaatcagtctcatgcgccattagcgctaggctagttagcgtggaggaccggagcgctaccgccagcagtttcatccgcctggttacgggtttgttaacacctaccggtgttttaccgctaccataggatccgatccatgggcggccgcggtac

SEQ ID NO: 23 - DNA, 6892 bp, Artificial Sequence
  Nucleotide sequence of transfer plasmid pU70-p455-H3-71K71
caataaacgcggtatgtctaccttcaagcctatgatgaacggatgtttggtgtttgcggctattataacgctcttgagttttatgctatctctgggaacatgcgaaaattacaggcgtgtggttcgggatcctagggataacagggtaatcgatttattcaacaaagccacgttgtgtctcaaaatctctgatgttacattgcacaagataaaaatatatcatcatgaacaataaaactgtctgcttacataaacagtaatacaaggggtgttatgagccatattcaacgggaaacgtcttgctcgaggccgcgattaaattccaacatggatgctgatttatatgggtataaatgggctcgcgataatgtcgggcaatcaggtgcgacaatctatcgattgtatgggaagcccgatgcgccagagttgtttctgaaacatggcaaaggtagcgttgccaatgatgttacagatgagatggtcagactaaactggctgacggaatttatgcctcttccgaccatcaagcattttatccgtactcctgatgatgcatggttactcaccactgcgatccccgggaaaacagcattccaggtattagaagaatatcctgattcaggtgaaaatattgttgatgcgctggcagtgttcctgcgccggttgcattcgattcctgtttgtaattgtccttttaacagcgatcgcgtatttcgtctcgctcaggcgcaatcacgaatgaataacggtttggttgatgcgagtgattttgatgacgagcgtaatggctggcctgttgaacaagtctggaaagaaatgcataagcttttgccattctcaccggattcagtcgtcactcatggtgatttctcacttgataaccttatttttgacgaggggaaattaataggttgtattgatgttggacgagtcggaatcgcagaccgataccaggatcttgccatcctatggaactgcctcggtgagttttctccttcattacagaaacggctttttcaaaaatatggtattgataatcctgatatgaataaattgcagtttcatttgatgctcgatgagtttttctaaaataaacgcggtatgtctaccttcaagcctatgatgaacggatgtttggtgtttgcggctattataacgctcttgagttttatgctatctctgggaacatgcgaaaattacaggcgtgtggttcgggatccgaccctgttggtgggtgcggttggactcagaatcttggcgcaggcatggaagtttgtcggtgacgaaacatacgacaccatccgcgcagaagcaaagaatttagagacccacgtaccctcaagtgctgcagagtcgtctctagaaaaccaatcgacacaggaggagtctaacagccccgaagttgcccacctgcgaagcgtcaacagcgatgacagtacacacacggggggtgcgtcgaacggcatccaggactgtgacagtcagctcaaaactgtgtatgcctgcttggctctaattggactcggcacatgtgccatgatagggttgatagtttacatttgtgtattaaggtcaaaactgtcctctcggaatttttcgcgcgcgcaaaatgtaaaacatagaaattaccagcgacttgagtacgttgcttaagcttggcgtaatcatggtcatagctgtttcctgtgtgaaattgttatccgctcacaattccacacaacatacgagccggaagcataaagtgtaaagcctggggtgcctaatgagtgagctaactcacattaattgcgttgcgctcactgcccgctttccagtcgggaaacctgtcgtgccagctgcattaatgaatcggccaacgcgcggggagaggcggtttgcgtattgggcgctcttccgcttcctcgctcactgactcgctgcgctcggtcgttcggctgcggcgagcggtatcagctcactcaaaggcggtaatacggttatccacagaatcaggggataacgcaggaaagaacatgtgagcaaaaggccagcaaaaggccaggaaccgtaaaaaggccgcgttgctggcgtttttccataggctccgcccccctgacgagcatcacaaaaatcgacgctcaagtcagaggtggcgaaacccgacaggactataaagataccaggcgtttccccctggaagctccctcgtgcgctctcctgttccgaccctgccgcttaccggatacctgtccgcctttctcccttcgggaagcgtggcgctttctcatagctcacgctgtaggtatctcagttcggtgtaggtcgttcgctccaagctgggctgtgtgcacgaaccccccgttcagcccgaccgctgcgccttatccggtaactatcgtcttgagtccaacccggtaagacacgacttatcgccactggcagcagccactggtaacaggattagcagagcgaggtatgtaggcggtgctacagagttcttgaagtggtggcctaactacggctacactagaaggacagtatttggtatctgcgctctgctgaagccagttaccttcggaaaaagagttggtagctcttgatccggcaaacaaaccaccgctggtagcggtggtttttttgtttgcaagcagcagattacgcgcagaaaaaaaggatctcaagaagatcctttgatcttttctacggggtctgacgctcagtggaacgaaaactcacgttaagggattttggtcatgagattatcaaaaaggatcttcacctagatccttttaaattaaaaatgaagttttaaatcaatctaaagtatatatgagtaaacttggtctgacagttaccaatgcttaatcagtgaggcacctatctcagcgatctgtctatttcgttcatccatagttgcctgactccccgtcgtgtagataactacgatacgggagggcttaccatctggccccagtgctgcaatgataccgcgagacccacgctcaccggctccagatttatcagcaataaaccagccagccggaagggccgagcgcagaagtggtcctgcaactttatccgcctccatccagtctattaattgttgccgggaagctagagtaagtagttcgccagttaatagtttgcgcaacgttgttgccattgctacaggcatcgtggtgtcacgctcgtcgtttggtatggcttcattcagctccggttcccaacgatcaaggcgagttacatgatcccccatgttgtgcaaaaaagcggttagctccttcggtcctccgatcgttgtcagaagtaagttggccgcagtgttatcactcatggttatggcagcactgcataattctcttactgtcatgccatccgtaagatgcttttctgtgactggtgagtactcaaccaagtcattctgagaatagtgtatgcggcgaccgagttgctcttgcccggcgtcaatacgggataataccgcgccacatagcagaactttaaaagtgctcatcattggaaaacgttcttcggggcgaaaactctcaaggatcttaccgctgttgagatccagttcgatgtaacccactcgtgcacccaactgatcttcagcatcttttactttcaccagcgtttctgggtgagcaaaaacaggaaggcaaaatgccgcaaaaaagggaataagggcgacacggaaatgttgaatactcatactcttcctttttcaatattattgaagcatttatcagggttattgtctcatgagcggatacatatttgaatgtatttagaaaaataaacaaataggggttccgcgcacatttccccgaaaagtgccacctgacgtctaagaaaccattattatcatgacattaacctataaaaataggcgtatcacgaggccctttcgtctcgcgcgtttcggtgatgacggtgaaaacctctgacacatgcagctcccggagacggtcacagcttgtctgtaagcggatgccgggagcagacaagcccgtcagggcgcgtcagcgggtgttggcgggtgtcggggctggcttaactatgcggcatcagagcagattgtactgagagtgcaccatatgcggtgtgaaataccgcacagatgcgtaaggagaaaataccgcatcaggcgccattcgccattcaggctgcgcaactgttgggaagggcgatcggtgcgggcctcttcgctattacgccagctggcgaaagggggatgtgctgcaaggcgattaagttgggtaacgccagggttttcccagtcacgacgttgtaaaacgacggccagtgaattcctccgagtaccccagaggagtatgtgaaaagctgccactcgcaactactgaagataatttcaacgctcaagataaatccggaggagtttcctcgagaccccgggtcgaggctcgtgcgcggatacatcgagtattctagactcgagcgcaagccctacacgcgctacccctgctttcaacgcgtcaacctgcacattgacggggagtttctggttcacaagatgctagcgttcaatgccgcgatgcgcccatcggccgaggagctgctgtcatacccaatgtttgctcaactttaggatgactaacctgtttctgggaggagacagcgtgggcgacggtgtataaagttggtctgctttcaagccctgccactgcgctacagtgccaccaactgtaaagcggtagtaagctgcagtggtcgactggtggtagcatatactaccttatttatacgctccgagctgtttttcagcatgctagcacccaacgccgagcgagagtatataactcccatcattgcccacaagcttatgccacttattagcgtccgctctgccgtttgcttagtcataatatctaccgccgtttacgcagcagacgctatctgcgacacaattggatttgcgataccgcgcatgtggatgtgtattttaatgagatcaacctccatgaagcgtaactagggggcctcccactgaggcactaccggcttagcagctgactaacacagtataaaacgtgagaagaaatcagtctcatgcgccattagcgctaggctagttagcgtggaggaccggagcgctaccgccagcagtttcatccgcctggttacgggtttgttaacacctaccggtgttttaccgctaccataggatccgatccatgggcggccgcatgaagaccgtgatcgccctgagttacatcttctgcctggtgtttgggcaggacctccctggtaaaggcaacaacacggccacgctgtgccttgggcaccacgccgtgccgaacggcacccttgtgaaaactattaccgacgatcagatcgaggtgaccaacgccaccgaactggttcagaattttagcatgggcaaaatttgcaataacccgcaccgcattctggacggggccaactgcacgctgatcgattcattgctgggtgatccccactgcgatggctttcaaaacgaaaagtgggacttgttcatcgaacgcagcaaggcattcagcaactgctacccatacgacgtgcccgaatacaccagcctgcgaagcctgatcgcgagctctgggaccctggagttcaccaatgagaacttcaattggaccggagtgacccaaaacggtggctccagcgcctgtaaaaggggacccaataacagcttctttagcaagttgaattggctttacaagagcggcaatacttacccgatgttgaatgtgaccatgcccaacagtgacgactttgataaactgtacatatggggcgtgcaccatcccagcacggaccgcgaacagataaacctgtacgtgcaggccagcgggaagataatcgtgagcaccaagcgcagccagcagaccatcattcccaacattggcagccgaccgtgggtgcgcggtctgagctcccgcatcagcatatactggaccattgtcaagccgggagacatcctgatcatcaactctaatggcaatcttatcgccccacgcggctacttcaagatgcagaccggcaaaagcagtgtgatgaggagcgacgcccccatcgacacctgcaatagcgaatgcatcacccccaatggcagcatccccaacgacaagcctttccagaacgtgaataagatcacctacggcgcgtgccccaagtacatcaagcagaacaccctgaagctggccaccggcatgcgcaacatccccgagcgacagacacggggcatttttggcgcaatcgcagggttcattgagaatggctgggagggaatggttaacggctggtacggcttccgccatcagaactctgaaggaatcggccaagctgcggatctgaagtccacgcaagcagccatcaaccagatcaacggcaagcttaaccgcgtgattgaaaagacgaacgagaaattccaccaaatagagaaagaattcagcgaggtggagggccgcatccaagacctcgagcgctacgtggaggacaccaagatcgacctgtggagctacaatgccgagctcctggtcgccttggaaaaccaacacaccattgacctgaccgacagcgagatgaataaactcttcgagaagacccggaagcaactccgagagaacgccgaagacatgggtaatgggtgttttaagatctaccacaagtgcgacaatagctgcatggagagcatccgaaacggaacctacgaccacaacgagtaccgcgatgaggcagttaataaccgcttccaaatcaaaagcgtggaactgaagagtggctataaggactggatactgtggatcagctttgccataagctgcttcctgctgtgcgccgtttggttgggtttcatcatgtgggcctgtcaaaagggcaatattcgctgtaacatctgcatttgaggtac

SEQ ID NO: 24 - DNA, 4977 bp, Artificial Sequence
  Nucleotide sequence of transfer vector pU-1-3-p430-BGHKBGH
cctgtgccttctagttgccagccatctgttgtttgcccctcccccgtgccttccttgaccctggaaggtgccactcccactgtcctttcctaataaaatgaggaaattgcatcgcattgtctgagtaggtgtcattctattctggggggtggggtggggcaggacagcaagggggaggattgggaagacaatagcaggcatgctggggatgcggtgggctctatggatcctagggataacagggtaatcgatttattcaacaaagccacgttgtgtctcaaaatctctgatgttacattgcacaagataaaaatatatcatcatgaacaataaaactgtctgcttacataaacagtaatacaaggggtgttatgagccatattcaacgggaaacgtcttgctcgaggccgcgattaaattccaacatggatgctgatttatatgggtataaatgggctcgcgataatgtcgggcaatcaggtgcgacaatctatcgattgtatgggaagcccgatgcgccagagttgtttctgaaacatggcaaaggtagcgttgccaatgatgttacagatgagatggtcagactaaactggctgacggaatttatgcctcttccgaccatcaagcattttatccgtactcctgatgatgcatggttactcaccactgcgatccccgggaaaacagcattccaggtattagaagaatatcctgattcaggtgaaaatattgttgatgcgctggcagtgttcctgcgccggttgcattcgattcctgtttgtaattgtccttttaacagcgatcgcgtatttcgtctcgctcaggcgcaatcacgaatgaataacggtttggttgatgcgagtgattttgatgacgagcgtaatggctggcctgttgaacaagtctggaaagaaatgcataagcttttgccattctcaccggattcagtcgtcactcatggtgatttctcacttgataaccttatttttgacgaggggaaattaataggttgtattgatgttggacgagtcggaatcgcagaccgataccaggatcttgccatcctatggaactgcctcggtgagttttctccttcattacagaaacggctttttcaaaaatatggtattgataatcctgatatgaataaattgcagtttcatttgatgctcgatgagtttttctaaccatggctgtgccttctagttgccagccatctgttgtttgcccctcccccgtgccttccttgaccctggaaggtgccactcccactgtcctttcctaataaaatgaggaaattgcatcgcattgtctgagtaggtgtcattctattctggggggtggggtggggcaggacagcaagggggaggattgggaagacaatagcaggcatgctggggatgcggtgggctctatggatccgaccctccccggggctaaaaagctgcgtcttcacgcccgaggcgcttattgcccactgggtacggggcgcgcttttatatgtgtaacgtcccaccggtgtgacgcacgtactacggttgttctaaatagctgtccccgtgattgcctcggctgcacacatcgcctaggtttccgccgtgcctggtgtcgagggcccacccctgtaaccaacatcgatgggggcctgctgctccttcgctaccttaggaccgttatagttacgtcaagcttggcgtaatcatggtcatagctgtttcctgtgtgaaattgttatccgctcacaattccacacaacatacgagccggaagcataaagtgtaaagcctggggtgcctaatgagtgagctaactcacattaattgcgttgcgctcactgcccgctttccagtcgggaaacctgtcgtgccagctgcattaatgaatcggccaacgcgcggggagaggcggtttgcgtattgggcgctcttccgcttcctcgctcactgactcgctgcgctcggtcgttcggctgcggcgagcggtatcagctcactcaaaggcggtaatacggttatccacagaatcaggggataacgcaggaaagaacatgtgagcaaaaggccagcaaaaggccaggaaccgtaaaaaggccgcgttgctggcgtttttccataggctccgcccccctgacgagcatcacaaaaatcgacgctcaagtcagaggtggcgaaacccgacaggactataaagataccaggcgtttccccctggaagctccctcgtgcgctctcctgttccgaccctgccgcttaccggatacctgtccgcctttctcccttcgggaagcgtggcgctttctcatagctcacgctgtaggtatctcagttcggtgtaggtcgttcgctccaagctgggctgtgtgcacgaaccccccgttcagcccgaccgctgcgccttatccggtaactatcgtcttgagtccaacccggtaagacacgacttatcgccactggcagcagccactggtaacaggattagcagagcgaggtatgtaggcggtgctacagagttcttgaagtggtggcctaactacggctacactagaaggacagtatttggtatctgcgctctgctgaagccagttaccttcggaaaaagagttggtagctcttgatccggcaaacaaaccaccgctggtagcggtggtttttttgtttgcaagcagcagattacgcgcagaaaaaaaggatctcaagaagatcctttgatcttttctacggggtctgacgctcagtggaacgaaaactcacgttaagggattttggtcatgagattatcaaaaaggatcttcacctagatccttttaaattaaaaatgaagttttaaatcaatctaaagtatatatgagtaaacttggtctgacagttaccaatgcttaatcagtgaggcacctatctcagcgatctgtctatttcgttcatccatagttgcctgactccccgtcgtgtagataactacgatacgggagggcttaccatctggccccagtgctgcaatgataccgcgagacccacgctcaccggctccagatttatcagcaataaaccagccagccggaagggccgagcgcagaagtggtcctgcaactttatccgcctccatccagtctattaattgttgccgggaagctagagtaagtagttcgccagttaatagtttgcgcaacgttgttgccattgctacaggcatcgtggtgtcacgctcgtcgtttggtatggcttcattcagctccggttcccaacgatcaaggcgagttacatgatcccccatgttgtgcaaaaaagcggttagctccttcggtcctccgatcgttgtcagaagtaagttggccgcagtgttatcactcatggttatggcagcactgcataattctcttactgtcatgccatccgtaagatgcttttctgtgactggtgagtactcaaccaagtcattctgagaatagtgtatgcggcgaccgagttgctcttgcccggcgtcaatacgggataataccgcgccacatagcagaactttaaaagtgctcatcattggaaaacgttcttcggggcgaaaactctcaaggatcttaccgctgttgagatccagttcgatgtaacccactcgtgcacccaactgatcttcagcatcttttactttcaccagcgtttctgggtgagcaaaaacaggaaggcaaaatgccgcaaaaaagggaataagggcgacacggaaatgttgaatactcatactcttcctttttcaatattattgaagcatttatcagggttattgtctcatgagcggatacatatttgaatgtatttagaaaaataaacaaataggggttccgcgcacatttccccgaaaagtgccacctgacgtctaagaaaccattattatcatgacattaacctataaaaataggcgtatcacgaggccctttcgtctcgcgcgtttcggtgatgacggtgaaaacctctgacacatgcagctcccggagacggtcacagcttgtctgtaagcggatgccgggagcagacaagcccgtcagggcgcgtcagcgggtgttggcgggtgtcggggctggcttaactatgcggcatcagagcagattgtactgagagtgcaccatatgcggtgtgaaataccgcacagatgcgtaaggagaaaataccgcatcaggcgccattcgccattcaggctgcgcaactgttgggaagggcgatcggtgcgggcctcttcgctattacgccagctggcgaaagggggatgtgctgcaaggcgattaagttgggtaacgccagggttttcccagtcacgacgttgtaaaacgacggccagtgaattcgacgtaactataacggtcctaaggtagcgaatttttccattgggcccctcccttttggctctgggtatttagcttccctcccacttctcattccactttctccacctgcaccttttccatctcctctccaactcgccgccatgagacccgagggagtttcgcggggccgcgcctcctctgtctccatctccaactagtgtcgacctctatttgaggacccgccgagtaccccacaagagtatgtaaaaagctgtcattctcaactactgagaataatatcaaagctaaagataaaccctgaggagtttccacgggaaccagagtctaggctcgtgcgcggatacatcgaatacgccagcctagagcgtaagccacatacgcgctatccttgcttccagcgcgtgaacctacacattgacggggaatttttgatccataaaatgctagcgttcaatgctgcgatgcgcccatccgcagaagagttgttgtcctacccaatgtttatgaatctgtaggatgactaacagatttggggtggagacggcgtgggcgatactgtataaagttgtactacttaccagcccagtcagtgtgctgtagtgccaccacctgtaaagctgtgataagctgcagttgcggccgccgggtac

SEQ ID NO: 25 - DNA, 6678 bp, Artificial Sequence
  Nucleotide sequence of transfer plasmid pU1-3-p430-H1av-BGHKBGH
cctgtgccttctagttgccagccatctgttgtttgcccctcccccgtgccttccttgaccctggaaggtgccactcccactgtcctttcctaataaaatgaggaaattgcatcgcattgtctgagtaggtgtcattctattctggggggtggggtggggcaggacagcaagggggaggattgggaagacaatagcaggcatgctggggatgcggtgggctctatggatcctagggataacagggtaatcgatttattcaacaaagccacgttgtgtctcaaaatctctgatgttacattgcacaagataaaaatatatcatcatgaacaataaaactgtctgcttacataaacagtaatacaaggggtgttatgagccatattcaacgggaaacgtcttgctcgaggccgcgattaaattccaacatggatgctgatttatatgggtataaatgggctcgcgataatgtcgggcaatcaggtgcgacaatctatcgattgtatgggaagcccgatgcgccagagttgtttctgaaacatggcaaaggtagcgttgccaatgatgttacagatgagatggtcagactaaactggctgacggaatttatgcctcttccgaccatcaagcattttatccgtactcctgatgatgcatggttactcaccactgcgatccccgggaaaacagcattccaggtattagaagaatatcctgattcaggtgaaaatattgttgatgcgctggcagtgttcctgcgccggttgcattcgattcctgtttgtaattgtccttttaacagcgatcgcgtatttcgtctcgctcaggcgcaatcacgaatgaataacggtttggttgatgcgagtgattttgatgacgagcgtaatggctggcctgttgaacaagtctggaaagaaatgcataagcttttgccattctcaccggattcagtcgtcactcatggtgatttctcacttgataaccttatttttgacgaggggaaattaataggttgtattgatgttggacgagtcggaatcgcagaccgataccaggatcttgccatcctatggaactgcctcggtgagttttctccttcattacagaaacggctttttcaaaaatatggtattgataatcctgatatgaataaattgcagtttcatttgatgctcgatgagtttttctaaccatggctgtgccttctagttgccagccatctgttgtttgcccctcccccgtgccttccttgaccctggaaggtgccactcccactgtcctttcctaataaaatgaggaaattgcatcgcattgtctgagtaggtgtcattctattctggggggtggggtggggcaggacagcaagggggaggattgggaagacaatagcaggcatgctggggatgcggtgggctctatggatccgaccctccccggggctaaaaagctgcgtcttcacgcccgaggcgcttattgcccactgggtacggggcgcgcttttatatgtgtaacgtcccaccggtgtgacgcacgtactacggttgttctaaatagctgtccccgtgattgcctcggctgcacacatcgcctaggtttccgccgtgcctggtgtcgagggcccacccctgtaaccaacatcgatgggggcctgctgctccttcgctaccttaggaccgttatagttacgtcaagcttggcgtaatcatggtcatagctgtttcctgtgtgaaattgttatccgctcacaattccacacaacatacgagccggaagcataaagtgtaaagcctggggtgcctaatgagtgagctaactcacattaattgcgttgcgctcactgcccgctttccagtcgggaaacctgtcgtgccagctgcattaatgaatcggccaacgcgcggggagaggcggtttgcgtattgggcgctcttccgcttcctcgctcactgactcgctgcgctcggtcgttcggctgcggcgagcggtatcagctcactcaaaggcggtaatacggttatccacagaatcaggggataacgcaggaaagaacatgtgagcaaaaggccagcaaaaggccaggaaccgtaaaaaggccgcgttgctggcgtttttccataggctccgcccccctgacgagcatcacaaaaatcgacgctcaagtcagaggtggcgaaacccgacaggactataaagataccaggcgtttccccctggaagctccctcgtgcgctctcctgttccgaccctgccgcttaccggatacctgtccgcctttctcccttcgggaagcgtggcgctttctcatagctcacgctgtaggtatctcagttcggtgtaggtcgttcgctccaagctgggctgtgtgcacgaaccccccgttcagcccgaccgctgcgccttatccggtaactatcgtcttgagtccaacccggtaagacacgacttatcgccactggcagcagccactggtaacaggattagcagagcgaggtatgtaggcggtgctacagagttcttgaagtggtggcctaactacggctacactagaaggacagtatttggtatctgcgctctgctgaagccagttaccttcggaaaaagagttggtagctcttgatccggcaaacaaaccaccgctggtagcggtggtttttttgtttgcaagcagcagattacgcgcagaaaaaaaggatctcaagaagatcctttgatcttttctacggggtctgacgctcagtggaacgaaaactcacgttaagggattttggtcatgagattatcaaaaaggatcttcacctagatccttttaaattaaaaatgaagttttaaatcaatctaaagtatatatgagtaaacttggtctgacagttaccaatgcttaatcagtgaggcacctatctcagcgatctgtctatttcgttcatccatagttgcctgactccccgtcgtgtagataactacgatacgggagggcttaccatctggccccagtgctgcaatgataccgcgagacccacgctcaccggctccagatttatcagcaataaaccagccagccggaagggccgagcgcagaagtggtcctgcaactttatccgcctccatccagtctattaattgttgccgggaagctagagtaagtagttcgccagttaatagtttgcgcaacgttgttgccattgctacaggcatcgtggtgtcacgctcgtcgtttggtatggcttcattcagctccggttcccaacgatcaaggcgagttacatgatcccccatgttgtgcaaaaaagcggttagctccttcggtcctccgatcgttgtcagaagtaagttggccgcagtgttatcactcatggttatggcagcactgcataattctcttactgtcatgccatccgtaagatgcttttctgtgactggtgagtactcaaccaagtcattctgagaatagtgtatgcggcgaccgagttgctcttgcccggcgtcaatacgggataataccgcgccacatagcagaactttaaaagtgctcatcattggaaaacgttcttcggggcgaaaactctcaaggatcttaccgctgttgagatccagttcgatgtaacccactcgtgcacccaactgatcttcagcatcttttactttcaccagcgtttctgggtgagcaaaaacaggaaggcaaaatgccgcaaaaaagggaataagggcgacacggaaatgttgaatactcatactcttcctttttcaatattattgaagcatttatcagggttattgtctcatgagcggatacatatttgaatgtatttagaaaaataaacaaataggggttccgcgcacatttccccgaaaagtgccacctgacgtctaagaaaccattattatcatgacattaacctataaaaataggcgtatcacgaggccctttcgtctcgcgcgtttcggtgatgacggtgaaaacctctgacacatgcagctcccggagacggtcacagcttgtctgtaagcggatgccgggagcagacaagcccgtcagggcgcgtcagcgggtgttggcgggtgtcggggctggcttaactatgcggcatcagagcagattgtactgagagtgcaccatatgcggtgtgaaataccgcacagatgcgtaaggagaaaataccgcatcaggcgccattcgccattcaggctgcgcaactgttgggaagggcgatcggtgcgggcctcttcgctattacgccagctggcgaaagggggatgtgctgcaaggcgattaagttgggtaacgccagggttttcccagtcacgacgttgtaaaacgacggccagtgaattcgacgtaactataacggtcctaaggtagcgaatttttccattgggcccctcccttttggctctgggtatttagcttccctcccacttctcattccactttctccacctgcaccttttccatctcctctccaactcgccgccatgagacccgagggagtttcgcggggccgcgcctcctctgtctccatctccaactagtgtcgacctctatttgaggacccgccgagtaccccacaagagtatgtaaaaagctgtcattctcaactactgagaataatatcaaagctaaagataaaccctgaggagtttccacgggaaccagagtctaggctcgtgcgcggatacatcgaatacgccagcctagagcgtaagccacatacgcgctatccttgcttccagcgcgtgaacctacacattgacggggaatttttgatccataaaatgctagcgttcaatgctgcgatgcgcccatccgcagaagagttgttgtcctacccaatgtttatgaatctgtaggatgactaacagatttggggtggagacggcgtgggcgatactgtataaagttgtactacttaccagcccagtcagtgtgctgtagtgccaccacctgtaaagctgtgataagctgcagttgcggccgccgatggaggcaaaattgttcgtgctgttctgcgccttcactgctctgaaggcagacaccatctgcgtgggttaccacgccaataattccaccgacacggtggataccatcctggagaagaacgtgaccgtgactcattccgtgaacctcttggagaactcacacaatggtaaattgtgcagccttaacggcaaagccccgctgcaattggggaattgtaacgtggccggatggatactggggaaccccgagtgcgaccttctcctgaccgccaacagttggtcctacatcattgagacgagcaacagcaagaatggcgcctgctatcctggggagttcgctgactacgaggagctgcgcgagcagttgtctacagtcagcagcttcgaaagattcgagatcttcccaaaggccactagctggcccaaccacgatactaccaagggcactacagtgagttgcagccacagcggtgccaatagcttctaccgcaacctgctgtggatcgtgaagaagggtaacagctaccccaagctgagcaaatcttacacaaacaacaaaggcaaagaggtgttggttatctggggcgtgcatcatcccccaaccgactccgatcagcaaaccctgtaccagaacaaccacacctacgtgagcgtcggtagctctaagtattaccagcgcttcacccccgaaatcgtcgcacgaccgaaggtgagagggcaggccgggagaatgaactactactggaccctgctggatcaaggcgacactattaccttcgaggctaccggcaacttgatcgccccgtggcacgcgttcgccctcaataaaggatctaatagcggcataatgatgagtgatgcccacgtgcataactgcaccacgaagtgccagacccctcacggcgcactgaaaagcaatctgccctttcagaatgtgcaccccatcaccatcggcgagtgccccaagtatgttaaaagcactcagctccgcatggccaccggactgcgcaacatcccgagcatccaatcccgcggactgttcggcgcaatcgcgggctttatagagggcggctggaccggcatgatcgacggctggtacggctaccaccatcaaaatgagcaaggttccggctacgccgcagaccagaagagcacccaaatagcaatcgatggcatctccaacaaggtgaacagcgtgatcgaaaagatgaacatccagttcacaagcgtggggaaggagttcaataacctggaaaagcgcatcgagaatctgaacaagaaggttgacgatgggttcctcgatgtctggacctataacgccgagctcctgatactgcttgagaacgagcgcaccctggacttccacgacttcaacgtgaaaaacctgtacgaaaaggtcaagtcacagttgcgaaacaatgcgaaggagataggcaacggctgcttcgagttctatcacaagtgtgacaacgagtgcatggagagcgtcaagaacggcacttacaactacccgcgctactctgaggagagtaagctcaaccgcgaagagattgacggcgtgaaactggaaagcgttggtgtccatcagatcctggccatctacagcaccgtggctagctctctggttctgttggtgagcctgggcgctataagcttttggatgtgttctaatgggagcctgcagtgccgcatctgcatctgaggtac

SEQ ID NO: 26 - protein, 566 aa, Influenza A virus
MKAILVVLLYTFATANADTLCIGYHANNSTDTVDTVLEKNVTVTHSVNLLEDKHNGKLCKLRGVAPLHLGKCNIAGWILGNPECESLSTASSWSYIVETSSSDNGTCYPGDFIDYEELREQLSSVSSFERFEIFPKTSSWPNHDSNKGVTAACPHAGAKSFYKNLIWLVKKGNSYPKLSKSYINDKGKEVLVLWGIHHPSTSADQQSLYQNADAYVFVGTSRYSKKFKPEIAIRPKVRDQEGRMNYYWTLVEPGDKITFEATGNLVVPRYAFAMERKAGSGIIISDTPVHDCNTTCQTPKGAINTSLPFQNIHPITIGKCPKYVKSTKLRLATGLRNIPSIQSRGLFGAIAGFIEGGWTGMVDGWYGYHHQNEQGSGYAADLKSTQNAIDEITNKVNSVIEKMNTQFTAVGKEFNHLEKRIENLNKKVDDGFLDIWTYNAELLVLLENERTLDYHDSNVKNLYEKVRSQLKNNAKEIGNGCFEFYHKCDNTCMESVKNGTYDYPKYSEEAKLNREEIDGVKLESTRIYQILAIYSTVASSLVLIVSLGAISFWMCSNGSLQCRICI

SEQ ID NO: 27 - protein, 566 aa, Influenza A virus
MKTVIALSYIFCLVFGQDLPGKGNNTATLCLGHHAVPNGTLVKTITDDQIEVTNATELVQNFSMGKICNNPHRILDGANCTLIDSLLGDPHCDGFQNEKWDLFIERSKAFSNCYPYDVPEYTSLRSLIASSGTLEFTNENFNWTGVTQNGGSSACKRGPNNSFFSKLNWLYKSGNTYPMLNVTMPNSDDFDKLYIWGVHHPSTDREQINLYVQASGKIIVSTKRSQQTIIPNIGSRPWVRGLSSRISIYWTIVKPGDILIINSNGNLIAPRGYFKMQTGKSSVMRSDAPIDTCNSECITPNGSIPNDKPFQNVNKITYGACPKYIKQNTLKLATGMRNIPERQTRGIFGAIAGFIENGWEGMVNGWYGFRHQNSEGIGQAADLKSTQAAINQINGKLNRVIEKTNEKFHQIEKEFSEVEGRIQDLERYVEDTKIDLWSYNAELLVALENQHTIDLTDSEMNKLFEKTRKQLRENAEDMGNGCFKIYHKCDNSCMESIRNGTYDHNEYRDEAVNNRFQIKSVELKSGYKDWILWISFAISCFLLCAVWLGFIMWACQKGNIRCNICI

SEQ ID NO: 28 - protein, 566 aa, Influenza A virus
MEAKLFVLFCAFTALKADTICVGYHANNSTDTVDTILEKNVTVTHSVNLLENSHNGKLCSLNGKAPLQLGNCNVAGWILGNPECDLLLTANSWSYIIETSNSKNGACYPGEFADYEELREQLSTVSSFERFEIFPKATSWPNHDTTKGTTVSCSHSGANSFYRNLLWIVKKGNSYPKLSKSYTNNKGKEVLVIWGVHHPPTDSDQQTLYQNNHTYVSVGSSKYYQRFTPEIVARPKVRGQAGRMNYYWTLLDQGDTITFEATGNLIAPWHAFALNKGSNSGIMMSDAHVHNCTTKCQTPHGALKSNLPFQNVHPITIGECPKYVKSTQLRMATGLRNIPSIQSRGLFGAIAGFIEGGWTGMIDGWYGYHHQNEQGSGYAADQKSTQIAIDGISNKVNSVIEKMNIQFTSVGKEFNNLEKRIENLNKKVDDGFLDVWTYNAELLILLENERTLDFHDFNVKNLYEKVKSQLRNNAKEIGNGCFEFYHKCDNECMESVKNGTYNYPRYSEESKLNREEIDGVKLESVGVHQILAIYSTVASSLVLLVSLGAISFWMCSNGSLQCRICI

SEQ ID NO: 29 - protein, 564 aa, Influenza A virus
MKAKLLILWCALSATDADTICIGYHANNSTDTVDTVLEKNVTVTHSVNLLEDNHNGKLCKLKGVAPLQLGKCSIAGWILGNPECESLFSKKSWSYIAETPNAENGICYPGYFSDYEELREQLSSVSSFERFEIFPKESSWPKHSIGATASCSKQGRSSFYRNLLWLTEKNGSYPNLSKSYVNDKEREVLVLWGVHHPSNIEDQRAIYRKETAYVSVMSSLYNRRFTPEIAKRPKIRNQEGRINYYWTLLEPKDTIIFEANGNLIAPWYAFALSRGFESGIIVSNASMDECDAKCQTPQGAINSSLPFQNVHPVTIGECPKYVKSTKLKMATGLRNIPSIQTRGLFGAIAGFIEGGWTGMIDGWYGYHHQNEQGSGYAADQKSTQNAINGITNKVNSVIDKMNTQFTAVGKEFNKLEKRMENLNKKVDDGFLDIWTYNAELLVLLENERTLDFHDSNVKSLYEKVKGQLKNNAKEIGNGCFEFYHKCNNECMDSVKNGTYDYPRYSEESKLNREKIDGVELKSMGVYQILAIYSTVASSLVLLVSLGATSFWMCSNGSLQCRICI

SEQ ID NO: 30 - protein, 19 aa, Artificial Sequence
  GS linker
HMGGSGGGGSGGGGSGGGT

SEQ ID NO: 31 - DNA, 947 bp, Artificial Sequence
  Synthesized DNA sequence of truncated glycoprotein c (Gc) including restriction sites for subcloning
gcggccgcatgaaggcgatcctggttgtgctgctgtacacctttgccaccgccaacgccgatacgctgatcaactgcaagaacatccagagcacccagctgacaatcgagcacctgagcaagtgcatggccttctaccagaacaagaccagcagccccgtcgtgatcaacgagatcatctccgacgccagcgtggacgaacaggaactgattaagtctctgaacctgaactgcaacgtgatcgaccggttcatcagcgagtccagcgtgatcgagacacaggtgtactacgagtatatcaagagccagctgtgtccactgcaagtgcacgatatcttcaccatcaacagcgccagcaacatccagtggaaggccctggcccgcagctttaccctgggcgtgtgcaacaccaacccccacaagcacatctgccggtgcctggaatccatgcagatgtgtaccagcaccaagaccgaccacgccagagagatgagcatctactacgacggccaccccgacagattcgagcacgacatgaagattatcctgaatatcatgcggtacatcgtgcccggcctgggcagagtgctgctggaccagatcaagcagaccaaggactaccaggccctgagacacatccagggcaagctgagccccaagtcccagagcaacctgcagctgaagggcttcctggaattcgtggacttcatcctgggcgccaacgtgaccattgagaaaaccccccagaccctgaccaccctgagcctgattcatatgggaggttccggaggtggaggttccggaggtggaggttccggaggtggcaccatactggccatttacagcacagttgcgagcagcctggtcctgatcgtgagcctgggtgctatatcattctggatgtgcagcaacggctctctccagtgccgcatctgtatctgaggtacc

SEQ ID NO: 32 - DNA, 3060 bp, Artificial Sequence
  DNA fragment used for RED recombination to generate pRacH-SE-70-455-SBVGc,
tctagactcgagcgcaagccctacacgcgctacccctgctttcaacgcgtcaacctgcacattgacggggagtttctggttcacaagatgctagcgttcaatgccgcgatgcgcccatcggccgaggagctgctgtcatacccaatgtttgctcaactttaggatgactaacctgtttctgggaggagacagcgtgggcgacggtgtataaagttggtctgctttcaagccctgccactgcgctacagtgccaccaactgtaaagcggtagtaagctgcagtggtcgactggtggtagcatatactaccttatttatacgctccgagctgtttttcagcatgctagcacccaacgccgagcgagagtatataactcccatcattgcccacaagcttatgccacttattagcgtccgctctgccgtttgcttagtcataatatctaccgccgtttacgcagcagacgctatctgcgacacaattggatttgcgataccgcgcatgtggatgtgtattttaatgagatcaacctccatgaagcgtaactagggggcctcccactgaggcactaccggcttagcagctgactaacacagtataaaacgtgagaagaaatcagtctcatgcgccattagcgctaggctagttagcgtggaggaccggagcgctaccgccagcagtttcatccgcctggttacgggtttgttaacacctaccggtgttttaccgctaccataggatccgatccatgggcggccgcatgaaggcgatcctggttgtgctgctgtacacctttgccaccgccaacgccgatacgctgatcaactgcaagaacatccagagcacccagctgacaatcgagcacctgagcaagtgcatggccttctaccagaacaagaccagcagccccgtcgtgatcaacgagatcatctccgacgccagcgtggacgaacaggaactgattaagtctctgaacctgaactgcaacgtgatcgaccggttcatcagcgagtccagcgtgatcgagacacaggtgtactacgagtatatcaagagccagctgtgtccactgcaagtgcacgatatcttcaccatcaacagcgccagcaacatccagtggaaggccctggcccgcagctttaccctgggcgtgtgcaacaccaacccccacaagcacatctgccggtgcctggaatccatgcagatgtgtaccagcaccaagaccgaccacgccagagagatgagcatctactacgacggccaccccgacagattcgagcacgacatgaagattatcctgaatatcatgcggtacatcgtgcccggcctgggcagagtgctgctggaccagatcaagcagaccaaggactaccaggccctgagacacatccagggcaagctgagccccaagtcccagagcaacctgcagctgaagggcttcctggaattcgtggacttcatcctgggcgccaacgtgaccattgagaaaaccccccagaccctgaccaccctgagcctgattcatatgggaggttccggaggtggaggttccggaggtggaggttccggaggtggcaccatactggccatttacagcacagttgcgagcagcctggtcctgatcgtgagcctgggtgctatatcattctggatgtgcagcaacggctctctccagtgccgcatctgtatctgaggtaccaataaacgcggtatgtctaccttcaagcctatgatgaacggatgtttggtgtttgcggctattataacgctcttgagttttatgctatctctgggaacatgcgaaaattacaggcgtgtggttcgggatcctagggataacagggtaatcgatttattcaacaaagccacgttgtgtctcaaaatctctgatgttacattgcacaagataaaaatatatcatcatgaacaataaaactgtctgcttacataaacagtaatacaaggggtgttatgagccatattcaacgggaaacgtcttgctcgaggccgcgattaaattccaacatggatgctgatttatatgggtataaatgggctcgcgataatgtcgggcaatcaggtgcgacaatctatcgattgtatgggaagcccgatgcgccagagttgtttctgaaacatggcaaaggtagcgttgccaatgatgttacagatgagatggtcagactaaactggctgacggaatttatgcctcttccgaccatcaagcattttatccgtactcctgatgatgcatggttactcaccactgcgatccccgggaaaacagcattccaggtattagaagaatatcctgattcaggtgaaaatattgttgatgcgctggcagtgttcctgcgccggttgcattcgattcctgtttgtaattgtccttttaacagcgatcgcgtatttcgtctcgctcaggcgcaatcacgaatgaataacggtttggttgatgcgagtgattttgatgacgagcgtaatggctggcctgttgaacaagtctggaaagaaatgcataagcttttgccattctcaccggattcagtcgtcactcatggtgatttctcacttgataaccttatttttgacgaggggaaattaataggttgtattgatgttggacgagtcggaatcgcagaccgataccaggatcttgccatcctatggaactgcctcggtgagttttctccttcattacagaaacggctttttcaaaaatatggtattgataatcctgatatgaataaattgcagtttcatttgatgctcgatgagtttttctaaaataaacgcggtatgtctaccttcaagcctatgatgaacggatgtttggtgtttgcggctattataacgctcttgagttttatgctatctctgggaacatgcgaaaattacaggcgtgtggttcgggatccgaccctgttggtgggtgcggttggactcagaatcttggcgcaggcatggaagtttgtcggtgacgaaacatacgacaccatccgcgcagaagcaaagaatttagagacccacgtaccctcaagtgctgcagagtcgtctaga

SEQ ID NO: 33 - DNA, 17 bp, Artificial Sequence
  primer
cgtgcgcggatacatcg

SEQ ID NO: 34 - DNA, 16 bp, Artificial Sequence
  primer
cgcttcgcaggtgggc

SEQ ID NO: 35 - DNA, 19 bp, Artificial Sequence
  primer
gactggtggtagcatatac

SEQ ID NO: 36 - DNA, 19 bp, Artificial Sequence
  primer
gatcaacgagatcatctcc

SEQ ID NO: 37 - DNA, 17 bp, Artificial Sequence
  primer
ctggagagagccgttgc